European Patent Specification EP 3 442 561 B1, published February 14, 2024. Title: ADENO-ASSOCIATED VIRUS VECTOR DELIVERY OF MICRORNA-29 AND MICRO-DYSTROPHIN TO TREAT MUSCULAR DYSTROPHY. Applicant: RESEARCH INSTITUTE AT NATIONWIDE CHILDREN'S HOSPITAL RODINO-KLAPAC, et al. The sequence listing filed with the application follows.

SEQUENCE LISTING (13 sequences)

SEQ ID NO: 1 - DNA, 5910 bp, Adeno-associated virus
  promoter (120)..(526): CMV promotor
  Intron (927)..(1087): EF1a intron
  misc_feature (1088)..(1375): shRNA-miR29-c
  misc_feature (1257)..(1284): miR-29c
  Intron (1380)..(1854): EF1a intron
  misc_feature (1896)..(2091): polyA
cagcagctgcgcgctcgctcgctcactgaggccgcccgggcaaagcccgggcgtcgggcgacctttggtcgcccggcctcagtgagcgagcgagcgcgcagagagggagtggggttaaactcgttacataacttacggtaaatggcccgcctggctgaccgcccaacgacccccgcccattgacgtcaataatgacgtatgttcccatagtaacgccaatagggactttccattgacgtcaatgggtggagtatttacggtaaactgcccacttggcagtacatcaagtgtatcatatgccaagtacgccccctattgacgtcaatgacggtaaatggcccgcctggcattatgcccagtacatgaccttatgggactttcctacttggcagtacatctacgtattagtcatcgctattaccatggtgatgcggttttggcagtacatcaatgggcgtggatagcggtttgactcacggggatttccaagtctccaccccattgacgtcaatgggagtttgttttggcaccaaaatcaacgggactttccaaaatgtcgtaacaactccgccccattgacgcaaatgggcggtaggcgtgtacggtgggaggtctatataagcagagctcgtttagtgaaccgtcagatcgcctggagacgccatccacgctgttttgacctccatagaagacaccgggaccgatccagcctccggactctagaggatccggtactcgaggaactgaaaaaccagaaagttaactggtaagtttagtctttttgtcttttatttcaggtcccggatccggtggtggtgcaaatcaaagaactgctcctcagtggatgttgcctttacttctaggcctgtacggaagtgttacttctgctctaaaagctgcggaattgtacccggggccgatccaccggtctttttcgcaacgggtttgccgccagaacacaggtaagtgccgtgtgtggttcccgcgggcggcgacggggcccgtgcgtcccagcgcacatgttcggcgaggcggggcctgcgagcgcggccaccgagaatcggacgggggtagtctcaagctggccggcctgtttgaatgaggcttcagtactttacagaatcgttgcctgcacatcttggaaacacttgctgggattacttcttcaggttaacccaacagaaggctcgagaaggtatattgctgttgacagtgagcgcaaccgatttcaaatggtgctagagtgaagccacagatgtctagcaccatttgaaatcggttatgcctactgcctcggaattcaaggggctactttaggagcaattatcttgtttactaaaactgaataccttgctatctctttgatacattggccggcctgctctggtgcctggcctcgcgccgccgtgtatcgccccgccctgggcggcaaggctggcccggtcggcaccagttgcgtgagcggaaagatggccgcttcccggccctgctgcagggagctcaaaatggaggacgcggcgctcgggagagcgggcgggtgagtcacccacacaaaggaaaagggcctttccgtcctcagccgtcgcttcatgtgactccacggagtaccgggcgccgtccaggcacctcgattagttctcgagcttttggagtacgtcgtctttaggttggggggaggggttttatgcgatggagtttccccacactgagtgggtggagactgaagttaggccagcttggcacttgatgtaattctccttggaatttgccctttttgagtttggatcttggttcattctcaagcctcagacagtggttcaaagtttttttcttccatttcaggtgtcgtgaaaagctagcgctaccggactcagatctcgagctcaagctgcggggatccagacatgataagatacattgatgagtttggacaaaccacaactagaatgcagtgaaaaaaatgctttatttgtgaaatttgtgatgctattgctttatttgtaaccattataagctgcaataaacaagttaacaacaacaattgcattcattttatgtttcaggttcagggggaggtgtgggaggttttttcactagtagcatggctacgtagataagtagcatggcgggttaatcattaactacaaggaacccctagtgatggagttggccactccctctctgcgcgctcgctcgctcactgaggccgggcgaccaaaggtcgcccgacgcccgggctttgcccgggcggcctcagtgagcgagcgagcgcgccagctggcgtaatagcgaagaggcccgcaccgatcgcccttcccaacagttgcgcagcctgaatggcgaatggaattccagacgattgagcgtcaaaatgtaggtatttccatgagcgtttttcctgttgcaatggctggcggtaatattgttctggatattaccagcaaggccgatagtttgagttcttctactcaggcaagtgatgttattactaatcaaagaagtattgcgacaacggttaatttgcgtgatggacagactcttttactcggtggcctcactgattataaaaacacttctcaggattctggcgtaccgttcctgtctaaaatccctttaatcggcctcctgtttagctcccgctctgattctaacgaggaaagcacgttatacgtgctcgtcaaagcaaccatagtacgcgccctgtagcggcgcattaagcgcggcgggtgtggtggttacgcgcagcgtgaccgctacacttgccagcgccctagcgcccgctcctttcgctttcttcccttcctttctcgccacgttcgccggctttccccgtcaagctctaaatcgggggctccctttagggttccgatttagtgctttacggcacctcgaccccaaaaaacttgattagggtgatggttcacgtagtgggccatcgccctgatagacggtttttcgccctttgacgttggagtccacgttctttaatagtggactcttgttccaaactggaacaacactcaaccctatctcggtctattcttttgatttataagggattttgccgatttcggcctattggttaaaaaatgagctgatttaacaaaaatttaacgcgaattttaacaaaatattaacgtttacaatttaaatatttgcttatacaatcttcctgtttttggggcttttctgattatcaaccggggtacatatgattgacatgctagttttacgattaccgttcatcgattctcttgtttgctccagactctcaggcaatgacctgatagcctttgtagagacctctcaaaaatagctaccctctccggcatgaatttatcagctagaacggttgaatatcatattgatggtgatttgactgtctccggcctttctcacccgtttgaatctttacctacacattactcaggcattgcatttaaaatatatgagggttctaaaaatttttatccttgcgttgaaataaaggcttctcccgcaaaagtattacagggtcataatgtttttggtacaaccgatttagctttatgctctgaggctttattgcttaattttgctaattctttgccttgcctgtatgatttattggatgttggaattcctgatgcggtattttctccttacgcatctgtgcggtatttcacaccgcatatggtgcactctcagtacaatctgctctgatgccgcatagttaagccagccccgacacccgccaacacccgctgacgcgccctgacgggcttgtctgctcccggcatccgcttacagacaagctgtgaccgtctccgggagctgcatgtgtcagaggttttcaccgtcatcaccgaaacgcgcgagacgaaagggcctcgtgatacgcctatttttataggttaatgtcatgataataatggtttcttagacgtcaggtggcacttttcggggaaatgtgcgcggaacccctatttgtttatttttctaaatacattcaaatatgtatccgctcatgagacaataaccctgataaatgcttcaataatattgaaaaaggaagagtatgagtattcaacatttccgtgtcgcccttattcccttttttgcggcattttgccttcctgtttttgctcacccagaaacgctggtgaaagtaaaagatgctgaagatcagttgggtgcacgagtgggttacatcgaactggatctcaacagcggtaagatccttgagagttttcgccccgaagaacgttttccaatgatgagcacttttaaagttctgctatgtggcgcggtattatcccgtattgacgccgggcaagagcaactcggtcgccgcatacactattctcagaatgacttggttgagtactcaccagtcacagaaaagcatcttacggatggcatgacagtaagagaattatgcagtgctgccataaccatgagtgataacactgcggccaacttacttctgacaacgatcggaggaccgaaggagctaaccgcttttttgcacaacatgggggatcatgtaactcgccttgatcgttgggaaccggagctgaatgaagccataccaaacgacgagcgtgacaccacgatgcctgtagcaatggcaacaacgttgcgcaaactattaactggcgaactacttactctagcttcccggcaacaattaatagactggatggaggcggataaagttgcaggaccacttctgcgctcggcccttccggctggctggtttattgctgataaatctggagccggtgagcgtgggtctcgcggtatcattgcagcactggggccagatggtaagccctcccgtatcgtagttatctacacgacggggagtcaggcaactatggatgaacgaaatagacagatcgctgagataggtgcctcactgattaagcattggtaactgtcagaccaagtttactcatatatactttagattgatttaaaacttcatttttaatttaaaaggatctaggtgaagatcctttttgataatctcatgaccaaaatcccttaacgtgagttttcgttccactgagcgtcagaccccgtagaaaagatcaaaggatcttcttgagatcctttttttctgcgcgtaatctgctgcttgcaaacaaaaaaaccaccgctaccagcggtggtttgtttgccggatcaagagctaccaactctttttccgaaggtaactggcttcagcagagcgcagataccaaatactgtccttctagtgtagccgtagttaggccaccacttcaagaactctgtagcaccgcctacatacctcgctctgctaatcctgttaccagtggctgctgccagtggcgataagtcgtgtcttaccgggttggactcaagacgatagttaccggataaggcgcagcggtcgggctgaacggggggttcgtgcacacagcccagcttggagcgaacgacctacaccgaactgagatacctacagcgtgagctatgagaaagcgccacgcttcccgaagggagaaaggcggacaggtatccggtaagcggcagggtcggaacaggagagcgcacgagggagcttccagggggaaacgcctggtatctttatagtcctgtcgggtttcgccacctctgacttgagcgtcgatttttgtgatgctcgtcaggggggcggagcctatggaaaaacgccagcaacgcggcctttttacggttcctggccttttgctggccttttgctcacatgttctttcctgcgttatcccctgattctgtggataaccgtattaccgcctttgagtgagctgataccgctcgccgcagccgaacgaccgagcgcagcgagtcagtgagcgaggaagcggaagagcgcccaatacgcaaaccgcctctccccgcgcgttggccgattcattaatg

SEQ ID NO: 2 - DNA, 296 bp, Artificial Sequence
  Synthetic oligonucleotide
  misc_feature (1)..(8): FSE-I cut site
  misc_feature (9)..(136): miR-30 backbone
  misc_feature (139)..(160): miR-29c target (sense) strand
  misc_feature (161)..(175): miR-29c target (sense) strand
  misc_feature (176)..(199): miR-30 stem loop
  misc_feature (200)..(288): miR-29c guide (antisense) strand
  misc_feature (289)..(296): miR-30 backbone
ggccggcctgtttgaatgaggcttcagtactttacagaatcgttgcctgcacatcttggaaacacttgctgggattacttcttcaggttaacccaacagaaggctcgagaaggtatattgctgttgacagtgagcgcaaccgatttcaaatggtgctagagtgaagccacagatgtctagcaccatttgaaatcggttatgcctactgcctcggaattcaaggggctactttaggagcaattatcttgtttactaaaactgaataccttgctatctctttgatacattggccggcc

SEQ ID NO: 3 - DNA, 22 bp, Artificial Sequence
  Synthetic oligonucleotide
accgatttcaaatggtgctaga

SEQ ID NO: 4 - DNA, 24 bp, Artificial Sequence
  Synthetic oligonucleotide
tctagcaccatttgaaatcggtta

SEQ ID NO: 5 - DNA, 15 bp, Artificial Sequence
  Synthetic oligonucleotide
gtgaagccacagatg

SEQ ID NO: 6 - RNA, 98 nt, Artificial Sequence
  Synthetic oligonucleotide
  misc_feature (1)..(19): miR-30 backbone
  misc_feature (20)..(42): miR-29c target (sense) strand
  misc_feature (43)..(57): miR-30 stem loop
  misc_feature (58)..(81): miR-29c guide (antisense) strand
  misc_feature (82)..(98): miR-30 backbone
ugcuguugacagugagcgcaaccgauuucaaauggugcuagagugaagccacagaugucuagcaccauuugaaaucgguuaugccuacugccucggaa

SEQ ID NO: 7 - DNA, 3581 bp, Homo sapiens
  CDS (1)..(3579)
atgctgtggtgggaggaggtggaggattgttatgaaagggaggacgtgcagaagaagacttttaccaagtgggtgaacgctcagttcagcaaatttgggaagcagcacatcgagaatctgttttccgacctgcaggatgggagacggctgctggatctgctggaaggactgactggccagaagctgcccaaagagaaggggagcactagggtgcacgccctgaacaacgtgaacaaagctctgagagtgctgcagaacaacaacgtggatctggtgaatattggcagtactgatatcgtggacgggaaccacaaactgacactgggcctgatctggaacattattctgcactggcaggtgaaaaatgtgatgaagaacatcatggccgggctgcagcagaccaattccgagaagatcctgctgtcttgggtgcggcagagcacccgcaactatccccaggtgaacgtgattaacttcactacatcctggagcgacgggctggccctgaatgctctgattcacagccacaggcctgatctgttcgactggaatagcgtggtgtgccagcagtctgccacacagcgcctggaacatgccttcaatatcgctcggtaccagctggggatcgaaaaactgctggacccagaggatgtggacactacatacccagataaaaagtctattctgatgtacattactagcctgttccaggtgctgccacagcaggtgtctattgaagccattcaggaggtggaaatgctgccccgcccccccaaagtgactaaagaggagcattttcagctgcatcatcagatgcattacagccagcagattaccgtgagcctggctcagggatatgagcgcaccagtagtccaaaaccacggttcaagtcctacgcttatacccaggctgcctacgtgacaactagcgaccctactagatccccctttccatcccagcacctggaggccccagaggacaagagctttgggtccagcctgatggaaagcgaggtgaatctggatcggtaccagacagccctggaggaggtgctgagctggctgctgagtgctgaagacacactgcaggcccagggcgaaatttccaatgacgtggaagtggtgaaggatcagttccacacacacgagggctatatgatggacctgacagctcaccaggggcgcgtgggcaatatcctgcagctgggctctaaactgatcggcaccgggaaactgagtgaggacgaggaaacagaagtgcaggagcagatgaacctgctgaacagccgctgggagtgtctgagagtggctagtatggagaagcagtccaacctgcaccgggtgctgatggacctgcagaaccagaaactgaaagagctgaacgactggctgacaaagactgaggaacgcacaaggaagatggaggaggagccactgggacccgacctggaggatctgaagagacaggtgcagcagcataaggtgctgcaggaggatctggaacaggagcaggtgcgggtgaactccctgacacatatggtggtggtggtggacgaatctagtggagatcacgccaccgccgccctggaggaacagctgaaggtgctgggggaccggtgggccaacatttgccggtggaccgaggacaggtgggtgctgctgcaggacatcctgctgaaatggcagaggctgaccgaggagcagtgtctgtttagtgcttggctgagcgagaaagaggacgccgtgaacaagatccacacaaccggctttaaggatcagaacgaaatgctgtctagcctgcagaaactggctgtgctgaaggccgatctggagaaaaagaagcagagcatgggcaaactgtatagcctgaaacaggacctgctgagcaccctgaagaacaagagcgtgacccagaagacagaagcctggctggataactttgcccgctgctgggacaacctggtgcagaaactggagaaaagtacagctcagatctctcaggctgtgaccacaacccagcctagcctgacccagacaaccgtgatggaaaccgtgaccaccgtgacaacccgcgaacagatcctggtgaaacatgcccaggaagagctgccacctccacctccccagaagaagagaaccctggagcggctgcaggagctgcaggaagccactgacgaactggacctgaagctgaggcaggccgaagtgattaaggggtcttggcagcctgtgggcgatctgctgattgattccctgcaggaccacctggaaaaggtgaaggctctgagaggcgaaattgctccactgaaggagaacgtgagtcatgtgaacgatctggctagacagctgacaacactgggcatccagctgagcccatacaatctgagcacactggaggacctgaataccaggtggaagctgctgcaggtggctgtggaagaccgggtgcggcagctgcatgaggcccatcgcgacttcggaccagccagccagcactttctgagcacatccgtgcaggggccctgggagagggccatttctcccaacaaggtgccctactatattaatcacgagacccagaccacttgttgggaccatcccaagatgacagaactgtaccagtccctggccgatctgaacaacgtgaggtttagcgcttacagaaccgctatgaagctgagacggctgcagaaggccctgtgcctggatctgctgtccctgtccgccgcctgcgatgccctggatcagcataatctgaagcagaacgatcagccaatggatatcctgcagatcatcaactgcctgaccactatctacgacaggctggagcaggagcacaacaacctggtgaacgtgcctctgtgcgtggatatgtgcctgaactggctgctgaacgtgtatgacactgggcgcaccggccggatcagagtgctgagttttaaaactgggattatctccctgtgtaaggcccacctggaggacaagtacaggtacctgttcaagcaggtggctagtagcactggattttgtgaccagcgccgcctgggactgctgctgcatgatagtatccagattcctagacagctgggagaggtggctagtttcggaggatctaacatcgaacccagcgtgcgcagctgtttccagtttgccaataacaaacctgaaatcgaggctgctctgttcctggattggatgcgcctggaaccacagagcatggtgtggctgcctgtgctgcacagagtggctgccgccgaaactgccaagcaccaggctaaatgcaacatctgcaaggaatgtcccattatcggctttcgctacaggagtctgaaacattttaactacgatatttgccagagctgcttcttttccggaagagtggccaaaggacacaagatgcactaccctatggtggaatattgcaccccaactacatctggcgaagatgtgcgcgattttgccaaggtgctgaagaataagtttcggactaagaggtacttcgccaagcacccccgcatggggtatctgccagtgcagacagtgctggaaggagacaatatggagaccgatacaatgtgagc

SEQ ID NO: 8 - protein, 1192 aa, Homo sapiens
MLWWEEVEDCYEREDVQKKTFTKWVNAQFSKFGKQHIENLFSDLQDGRRLLDLLEGLTGQKLPKEKGSTRVHALNNVNKALRVLQNNNVDLVNIGSTDIVDGNHKLTLGLIWNIILHWQVKNVMKNIMAGLQQTNSEKILLSWVRQSTRNYPQVNVINFTTSWSDGLALNALIHSHRPDLFDWNSVVCQQSATQRLEHAFNIARYQLGIEKLLDPEDVDTTYPDKKSILMYITSLFQVLPQQVSIEAIQEVEMLPRPPKVTKEEHFQLHHQMHYSQQITVSLAQGYERTSSPKPRFKSYAYTQAAYVTTSDPTRSPFPSQHLEAPEDKSFGSSLMESEVNLDRYQTALEEVLSWLLSAEDTLQAQGEISNDVEVVKDQFHTHEGYMMDLTAHQGRVGNILQLGSKLIGTGKLSEDEETEVQEQMNLLNSRWECLRVASMEKQSNLHRVLMDLQNQKLKELNDWLTKTEERTRKMEEEPLGPDLEDLKRQVQQHKVLQEDLEQEQVRVNSLTHMVVVVDESSGDHATAALEEQLKVLGDRWANICRWTEDRWVLLQDILLKWQRLTEEQCLFSAWLSEKEDAVNKIHTTGFKDQNEMLSSLQKLAVLKADLEKKKQSMGKLYSLKQDLLSTLKNKSVTQKTEAWLDNFARCWDNLVQKLEKSTAQISQAVTTTQPSLTQTTVMETVTTVTTREQILVKHAQEELPPPPPQKKRTLERLQELQEATDELDLKLRQAEVIKGSWQPVGDLLIDSLQDHLEKVKALRGEIAPLKENVSHVNDLARQLTTLGIQLSPYNLSTLEDLNTRWKLLQVAVEDRVRQLHEAHRDFGPASQHFLSTSVQGPWERAISPNKVPYYINHETQTTCWDHPKMTELYQSLADLNNVRFSAYRTAMKLRRLQKALCLDLLSLSAACDALDQHNLKQNDQPMDILQIINCLTTIYDRLEQEHNNLVNVPLCVDMCLNWLLNVYDTGRTGRIRVLSFKTGIISLCKAHLEDKYRYLFKQVASSTGFCDQRRLGLLLHDSIQIPRQLGEVASFGGSNIEPSVRSCFQFANNKPEIEAALFLDWMRLEPQSMVWLPVLHRVAAAETAKHQAKCNICKECPIIGFRYRSLKHFNYDICQSCFFSGRVAKGHKMHYPMVEYCTPTTSGEDVRDFAKVLKNKFRTKRYFAKHPRMGYLPVQTVLEGDNMETDTM

SEQ ID NO: 9 - DNA, 8409 bp, Adeno-associated virus
  promoter (236)..(799): MCK promotor
  Intron (844)..(993): Chimeric intron sequence
  misc_feature (1004)..(4584): Human Dystrophin sequence
  misc_feature (4585)..(4640): Poly A tail
  misc_feature (6606)..(7466): Ampicillin resistance
  misc_feature (7621)..(8240): pGEX plasmid backbone with pBR322 origin or replication
gcccaatacgcaaaccgcctctccccgcgcgttggccgattcattaatgcagctggcgcgctcgctcgctcactgaggccgcccgggcaaagcccgggcgtcgggcgacctttggtcgcccggcctcagtgagcgagcgagcgcgcagagagggagtggccaactccatcactaggggttccttgtagttaatgattaacccgccatgctaattatctacgtagccatgtctagacagccactatgggtctaggctgcccatgtaaggaggcaaggcctggggacacccgagatgcctggttataattaacccagacatgtggctgctccccccccccaacacctgctgcctgagcctcacccccaccccggtgcctgggtcttaggctctgtacaccatggaggagaagctcgctctaaaaataaccctgtccctggtgggctgtgggggactgagggcaggctgtaacaggcttgggggccagggcttatacgtgcctgggactcccaaagtattactgttccatgttcccggcgaagggccagctgtcccccgccagctagactcagcacttagtttaggaaccagtgagcaagtcagcccttggggcagcccatacaaggccatggggctgggcaagctgcacgcctgggtccggggtgggcacggtgcccgggcaacgagctgaaagctcatctgctctcaggggcccctccctggggacagcccctcctggctagtcacaccctgtaggctcctctatataacccaggggcacaggggctgcccccgggtcaccaccacctccacagcacagacagacactcaggagccagccagccaggtaagtttagtctttttgtcttttatttcaggtcccggatccggtggtggtgcaaatcaaagaactgctcctcagtggatgttgcctttacttctaggcctgtacggaagtgttacttctgctctaaaagctgcggaattgtacccgcggccgccaccatgctgtggtgggaggaggtggaggattgttatgaaagggaggacgtgcagaagaagacttttaccaagtgggtgaacgctcagttcagcaaatttgggaagcagcacatcgagaatctgttttccgacctgcaggatgggagacggctgctggatctgctggaaggactgactggccagaagctgcccaaagagaaggggagcactagggtgcacgccctgaacaacgtgaacaaagctctgagagtgctgcagaacaacaacgtggatctggtgaatattggcagtactgatatcgtggacgggaaccacaaactgacactgggcctgatctggaacattattctgcactggcaggtgaaaaatgtgatgaagaacatcatggccgggctgcagcagaccaattccgagaagatcctgctgtcttgggtgcggcagagcacccgcaactatccccaggtgaacgtgattaacttcactacatcctggagcgacgggctggccctgaatgctctgattcacagccacaggcctgatctgttcgactggaatagcgtggtgtgccagcagtctgccacacagcgcctggaacatgccttcaatatcgctcggtaccagctggggatcgaaaaactgctggacccagaggatgtggacactacatacccagataaaaagtctattctgatgtacattactagcctgttccaggtgctgccacagcaggtgtctattgaagccattcaggaggtggaaatgctgccccgcccccccaaagtgactaaagaggagcattttcagctgcatcatcagatgcattacagccagcagattaccgtgagcctggctcagggatatgagcgcaccagtagtccaaaaccacggttcaagtcctacgcttatacccaggctgcctacgtgacaactagcgaccctactagatccccctttccatcccagcacctggaggccccagaggacaagagctttgggtccagcctgatggaaagcgaggtgaatctggatcggtaccagacagccctggaggaggtgctgagctggctgctgagtgctgaagacacactgcaggcccagggcgaaatttccaatgacgtggaagtggtgaaggatcagttccacacacacgagggctatatgatggacctgacagctcaccaggggcgcgtgggcaatatcctgcagctgggctctaaactgatcggcaccgggaaactgagtgaggacgaggaaacagaagtgcaggagcagatgaacctgctgaacagccgctgggagtgtctgagagtggctagtatggagaagcagtccaacctgcaccgggtgctgatggacctgcagaaccagaaactgaaagagctgaacgactggctgacaaagactgaggaacgcacaaggaagatggaggaggagccactgggacccgacctggaggatctgaagagacaggtgcagcagcataaggtgctgcaggaggatctggaacaggagcaggtgcgggtgaactccctgacacatatggtggtggtggtggacgaatctagtggagatcacgccaccgccgccctggaggaacagctgaaggtgctgggggaccggtgggccaacatttgccggtggaccgaggacaggtgggtgctgctgcaggacatcctgctgaaatggcagaggctgaccgaggagcagtgtctgtttagtgcttggctgagcgagaaagaggacgccgtgaacaagatccacacaaccggctttaaggatcagaacgaaatgctgtctagcctgcagaaactggctgtgctgaaggccgatctggagaaaaagaagcagagcatgggcaaactgtatagcctgaaacaggacctgctgagcaccctgaagaacaagagcgtgacccagaagacagaagcctggctggataactttgcccgctgctgggacaacctggtgcagaaactggagaaaagtacagctcagatctctcaggctgtgaccacaacccagcctagcctgacccagacaaccgtgatggaaaccgtgaccaccgtgacaacccgcgaacagatcctggtgaaacatgcccaggaagagctgccacctccacctccccagaagaagagaaccctggagcggctgcaggagctgcaggaagccactgacgaactggacctgaagctgaggcaggccgaagtgattaaggggtcttggcagcctgtgggcgatctgctgattgattccctgcaggaccacctggaaaaggtgaaggctctgagaggcgaaattgctccactgaaggagaacgtgagtcatgtgaacgatctggctagacagctgacaacactgggcatccagctgagcccatacaatctgagcacactggaggacctgaataccaggtggaagctgctgcaggtggctgtggaagaccgggtgcggcagctgcatgaggcccatcgcgacttcggaccagccagccagcactttctgagcacatccgtgcaggggccctgggagagggccatttctcccaacaaggtgccctactatattaatcacgagacccagaccacttgttgggaccatcccaagatgacagaactgtaccagtccctggccgatctgaacaacgtgaggtttagcgcttacagaaccgctatgaagctgagacggctgcagaaggccctgtgcctggatctgctgtccctgtccgccgcctgcgatgccctggatcagcataatctgaagcagaacgatcagccaatggatatcctgcagatcatcaactgcctgaccactatctacgacaggctggagcaggagcacaacaacctggtgaacgtgcctctgtgcgtggatatgtgcctgaactggctgctgaacgtgtatgacactgggcgcaccggccggatcagagtgctgagttttaaaactgggattatctccctgtgtaaggcccacctggaggacaagtacaggtacctgttcaagcaggtggctagtagcactggattttgtgaccagcgccgcctgggactgctgctgcatgatagtatccagattcctagacagctgggagaggtggctagtttcggaggatctaacatcgaacccagcgtgcgcagctgtttccagtttgccaataacaaacctgaaatcgaggctgctctgttcctggattggatgcgcctggaaccacagagcatggtgtggctgcctgtgctgcacagagtggctgccgccgaaactgccaagcaccaggctaaatgcaacatctgcaaggaatgtcccattatcggctttcgctacaggagtctgaaacattttaactacgatatttgccagagctgcttcttttccggaagagtggccaaaggacacaagatgcactaccctatggtggaatattgcaccccaactacatctggcgaagatgtgcgcgattttgccaaggtgctgaagaataagtttcggactaagaggtacttcgccaagcacccccgcatggggtatctgccagtgcagacagtgctggaaggagacaatatggagaccgatacaatgtgagcggccgcaataaaagatctttattttcattagatctgtgtgttggttttttgtgtgtctagagcatggctacgtagataagtagcatggcgggttaatcattaactacaaggaacccctagtgatggagttggccactccctctctgcgcgctcgctcgctcactgaggccgggcgaccaaaggtcgcccgacgcccgggctttgcccgggcggcctcagtgagcgagcgagcgcgccagctggcgtaatagcgaagaggcccgcaccgatcgcccttcccaacagttgcgcagcctgaatggcgaatggaagttccagacgattgagcgtcaaaatgtaggtatttccatgagcgtttttcctgttgcaatggctggcggtaatattgttctggatattaccagcaaggccgatagtttgagttcttctactcaggcaagtgatgttattactaatcaaagaagtattgcgacaacggttaatttgcgtgatggacagactcttttactcggtggcctcactgattataaaaacacttctcaggattctggcgtaccgttcctgtctaaaatccctttaatcggcctcctgtttagctcccgctctgattctaacgaggaaagcacgttatacgtgctcgtcaaagcaaccatagtacgcgccctgtagcggcgcattaagcgcggcgggtgtggtggttacgcgcagcgtgaccgctacacttgccagcgccctagcgcccgctcctttcgctttcttcccttcctttctcgccacgttcgccggctttccccgtcaagctctaaatcgggggctccctttagggttccgatttagtgatttacggcacctcgaccccaaaaaacttgattagggtgatggttcacgtagtgggccatcgccctgatagacggtttttcgccctttgacgttggagtccacgttctttaatagtggactcttgttccaaactggaacaacactcaaccctatctcggtctattcttttgatttataagggattttgccgatttcggcctattggttaaaaaatgagctgatttaacaaaaatttaacgcgaattttaacaaaatattaacgtttacaatttaaatatttgcttatacaatcttcctgtttttggggcttttctgattatcaaccggggtacatatgattgacatgctagttttacgattaccgttcatcgattctcttgtttgctccagactctcaggcaatgacctgatagcctttgtagagacctctcaaaaatagctaccctctccggcatgaatttatcagctagaacggttgaatatcatattgatggtgatttgactgtctccggcctttctcacccgtttgaatctttacctacacattactcaggcattgcatttaaaatatatgagggttctaaaaatttttatccttgcgttgaaataaaggcttctcccgcaaaagtattacagggtcataatgtttttggtacaaccgatttagctttatgctctgaggctttattgcttaattttgctaattctttgccttgcctgtatgatttattggatgttggaagttcctgatgcggtattttctccttacgcatctgtgcggtatttcacaccgcatatggtgcactctcagtacaatctgctctgatgccgcatagttaagccagccccgacacccgccaacacccgctgacgcgccctgacgggcttgtctgctcccggcatccgcttacagacaagctgtgaccgtctccgggagctgcatgtgtcagaggttttcaccgtcatcaccgaaacgcgcgagacgaaagggcctcgtgatacgcctatttttataggttaatgtcatgataataatggtttcttagacgtcaggtggcacttttcggggaaatgtgcgcggaacccctatttgtttatttttctaaatacattcaaatatgtatccgctcatgagacaataaccctgataaatgcttcaataatattgaaaaaggaagagtatgagtattcaacatttccgtgtcgcccttattcccttttttgcggcattttgccttcctgtttttgctcacccagaaacgctggtgaaagtaaaagatgctgaagatcagttgggtgcacgagtgggttacatcgaactggatctcaacagcggtaagatccttgagagttttcgccccgaagaacgttttccaatgatgagcacttttaaagttctgctatgtggcgcggtattatcccgtattgacgccgggcaagagcaactcggtcgccgcatacactattctcagaatgacttggttgagtactcaccagtcacagaaaagcatcttacggatggcatgacagtaagagaattatgcagtgctgccataaccatgagtgataacactgcggccaacttacttctgacaacgatcggaggaccgaaggagctaaccgcttttttgcacaacatgggggatcatgtaactcgccttgatcgttgggaaccggagctgaatgaagccataccaaacgacgagcgtgacaccacgatgcctgtagcaatggcaacaacgttgcgcaaactattaactggcgaactacttactctagcttcccggcaacaattaatagactggatggaggcggataaagttgcaggaccacttctgcgctcggcccttccggctggctggtttattgctgataaatctggagccggtgagcgtgggtctcgcggtatcattgcagcactggggccagatggtaagccctcccgtatcgtagttatctacacgacggggagtcaggcaactatggatgaacgaaatagacagatcgctgagataggtgcctcactgattaagcattggtaactgtcagaccaagtttactcatatatactttagattgatttaaaacttcatttttaatttaaaaggatctaggtgaagatcctttttgataatctcatgaccaaaatcccttaacgtgagttttcgttccactgagcgtcagaccccgtagaaaagatcaaaggatcttcttgagatcctttttttctgcgcgtaatctgctgcttgcaaacaaaaaaaccaccgctaccagcggtggtttgtttgccggatcaagagctaccaactctttttccgaaggtaactggcttcagcagagcgcagataccaaatactgtccttctagtgtagccgtagttaggccaccacttcaagaactctgtagcaccgcgtacatacctcgctctgctaatcctgttaccagtggctgctgccagtggcgataagtcgtgtcttaccgggttggactcaagacgatagttaccggataaggcgcagcggtcgggctgaacggggggttcgtgcacacagcccagcttggagcgaacgacctacaccgaactgagatacctacagcgtgagctatgagaaagcgccacgcttcccgaagggagaaaggcggacaggtatccggtaagcggcagggtcggaacaggagagcgcacgagggagcttccagggggaaacgcctggtatctttatagtcctgtcgggtttcgccacctctgacttgagcgtcgatttttgtgatgctcgtcaggggggcggagcctatggaaaaacgccagcaacgcggcctttttacggttcctggccttttgctggccttttgctcacatgttctttcctgcgttatcccctgattctgtggataaccgtattaccgggtttgagtgagctgataccgctcgccgcagccgaacgaccgagcgcagcgagtcagtgagcgaccaagcggaagagc

SEQ ID NO: 10 - DNA, 206 bp, Artificial Sequence
  Synthetic oligonucleotide
  enhancer (1)..(206): MCK enhancer
cagccactatgggtctaggctgcccatgtaaggaggcaaggcctggggacacccgagatgcctggttataattaacccagacatgtggctgctccccccccccaacacctgctgcctgagcctcacccccaccccggtgcctgggtcttaggctctgtacaccatggaggagaagctcgctctaaaaataaccctgtccctggtgg

SEQ ID NO: 11 - DNA, 358 bp, Artificial Sequence
  Synthetic oligonucleotide
  promoter (1)..(358): MCK promoter
gctgtgggggactgagggcaggctgtaacaggcttgggggccagggcttatacgtgcctgggactcccaaagtattactgttccatgttcccggcgaagggccagctgtcccccgccagctagactcagcacttagtttaggaaccagtgagcaagtcagcccttggggcagcccatacaaggccatggggctgggcaagctgcacgcctgggtccggggtgggcacggtgcccgggcaacgagctgaaagctcatctgctctcaggggcccctccctggggacagcccctcctggctagtcacaccctgtaggctcctctatataacccaggggcacaggggctgcccccgggtcac

SEQ ID NO: 12 - DNA, 5920 bp, Adeno-associated virus
  misc_feature: pAAV.MCK.miR26C Sequence
  misc_feature (4)..(9): n is a, c, g, t or u
  enhancer (190)..(395): MCK enhancer
  promoter (396)..(753): MCK promoter
  misc_feature (1316)..(1608): shRNA-miR29-c with primary seed sequence
  misc_feature (1487)..(1512): miR-29c
  misc_feature (2094)..(2146): SV40 PolyA
  misc_feature (2326)..(2331): n is a, c, g, t or u
ctgnnnnnngcgcgctcgctcgctcactgaggccgcccgggcaaagcccgggcgtcgggcgacctttggtcgcccggcctcagtgagcgagcgagcgcgcagagagggagtggccaactccatcactaggggttccttgtagttaatgattaacccgccatgctaattatctacgtagccatgtctagacagccactatgggtctaggctgcccatgtaaggaggcaaggcctggggacacccgagatgcctggttataattaacccagacatgtggctgctccccccccccaacacctgctgcctgagcctcacccccaccccggtgcctgggtcttaggctctgtacaccatggaggagaagctcgctctaaaaataaccctgtccctggtgggctgtgggggactgagggcaggctgtaacaggcttgggggccagggcttatacgtgcctgggactcccaaagtattactgttccatgttcccggcgaagggccagctgtcccccgccagctagactcagcacttagtttaggaaccagtgagcaagtcagcccttggggcagcccatacaaggccatggggctgggcaagctgcacgcctgggtccggggtgggcacggtgcccgggcaacgagctgaaagctcatctgctctcaggggcccctccctggggacagcccctcctggctagtcacaccctgtaggctcctctatataacccaggggcacaggggctgcccccgggtcaccaccacctccacagcacagacagacactcaggagccagccagccaggtaagtttagtctttttgtcttttatttcaggtcccggatccggtggtggtgcaaatcaaagaactgctcctcagtggatgttgcctttacttctaggcctgtacggaagtgttacttctgctctaaaagctgcggaattgtacccgcctagaggatccggtactcgaggaactgaaaaaccagaaagttaactggtaagtttagtctttttgtcttttatttcaggtcccggatccggtggtggtgcaaatcaaagaactgctcctcagtggatgttgcctttacttctaggcctgtacggaagtgttacttctgctctaaaagctgcggaattgtacccggggccgatccaccggtctttttcgcaacgggtttgccgccagaacacaggtaagtgccgtgtgtggttcccgcgggcggcgacggggcccgtgcgtcccagcgcacatgttcggcgaggcggggcctgcgagcgcggccaccgagaatcggacgggggtagtctcaagctggccggcctgtttgaatgaggcttcagtactttacagaatcgttgcctgcacatcttggaaacacttgctgggattacttcttcaggttaacccaacagaaggctcgagaaggtatattgctgttgacagtgagcgcaaccgatttcaaatggtgctagagtgaagccacagatgtctagcaccatttgaaatcggttatgcctactgcctcggaattcaaggggctactttaggagcaattatcttgtttactaaaactgaataccttgctatctctttgatacattggccggcctgctctggtgcctggcctcgcgccgccgtgtatcgccccgccctgggcggcaaggctggcccggtcggcaccagttgcgtgagcggaaagatggccgcttcccggccctgctgcagggagctcaaaatggaggacgcggcgctcgggagagcgggcgggtgagtcacccacacaaaggaaaagggcctttccgtcctcagccgtcgcttcatgtgactccacggagtaccgggcgccgtccaggcacctcgattagttctcgagcttttggagtacgtcgtctttaggttggggggaggggttttatgcgatggagtttccccacactgagtgggtggagactgaagttaggccagcttggcacttgatgtaattctccttggaatttgccctttttgagtttggatcttggttcattctcaagcctcagacagtggttcaaagtttttttcttccatttcaggtgtcgtgaaaagctagtgcggccgcaataaaagatctttattttcattagatctgtgtgttggttttttgtgtgtctagacatggctacgtagataattagcatggcgggttaatcattaactacaaggaacccctagtgatggagttggccactccctctctgcgcgctcgctcgctcactgaggccgggcgaccaaaggtcgcccgacgcccgggctttgcccgggcggcctcagtgagcgagcgagcgcgcnnnnnncagctggcgtaatagcgaagaggcccgcaccgatcgcccttcccaacagttgcgcagcctgaatggcgaatggaagttccagacgattgagcgtcaaaatgtaggtatttccatgagcgtttttcctgttgcaatggctggcggtaatattgttctggatattaccagcaaggccgatagtttgagttcttctactcaggcaagtgatgttattactaatcaaagaagtattgcgacaacggttaatttgcgtgatggacagactcttttactcggtggcctcactgattataaaaacacttctcaggattctggcgtaccgttcctgtctaaaatccctttaatcggcctcctgtttagctcccgctctgattctaacgaggaaagcacgttatacgtgctcgtcaaagcaaccatagtacgcgccctgtagcggcgcattaagcgcggcgggtgtggtggttacgcgcagcgtgaccgctacacttgccagcgccctagcgcccgctcctttcgctttcttcccttcctttctcgccacgttcgccggctttccccgtcaagctctaaatcgggggctccctttagggttccgatttagtgatttacggcacctcgaccccaaaaaacttgattagggtgatggttcacgtagtgggccatcgccctgatagacggtttttcgccctttgacgttggagtccacgttctttaatagtggactcttgttccaaactggaacaacactcaaccctatctcggtctattcttttgatttataagggattttgccgatttcggcctattggttaaaaaatgagctgatttaacaaaaatttaacgcgaattttaacaaaatattaacgtttacaatttaaatatttgcttatacaatcttcctgtttttggggcttttctgattatcaaccggggtacatatgattgacatgctagttttacgattaccgttcatcgattctcttgtttgctccagactctcaggcaatgacctgatagcctttgtagagacctctcaaaaatagctaccctctccggcatgaatttatcagctagaacggttgaatatcatattgatggtgatttgactgtctccggcctttctcacccgtttgaatctttacctacacattactcaggcattgcatttaaaatatatgagggttctaaaaatttttatccttgcgttgaaataaaggcttctcccgcaaaagtattacagggtcataatgtttttggtacaaccgatttagctttatgctctgaggctttattgcttaattttgctaattctttgccttgcctgtatgatttattggatgttggaagttcctgatgcggtattttctccttacgcatctgtgcggtatttcacaccgcatatggtgcactctcagtacaatctgctctgatgccgcatagttaagccagccccgacacccgccaacacccgctgacgcgccctgacgggcttgtctgctcccggcatccgcttacagacaagctgtgaccgtctccgggagctgcatgtgtcagaggttttcaccgtcatcaccgaaacgcgcgagacgaaagggcctcgtgatacgcctatttttataggttaatgtcatgataataatggtttcttagacgtcaggtggcacttttcggggaaatgtgcgcggaacccctatttgtttatttttctaaatacattcaaatatgtatccgctcatgagacaataaccctgataaatgcttcaataatattgaaaaaggaagagtatgagtattcaacatttccgtgtcgcccttattcccttttttgcggcattttgccttcctgtttttgctcacccagaaacgctggtgaaagtaaaagatgctgaagatcagttgggtgcacgagtgggttacatcgaactggatctcaacagcggtaagatccttgagagttttcgccccgaagaacgttttccaatgatgagcacttttaaagttctgctatgtggcgcggtattatcccgtattgacgccgggcaagagcaactcggtcgccgcatacactattctcagaatgacttggttgagtactcaccagtcacagaaaagcatcttacggatggcatgacagtaagagaattatgcagtgctgccataaccatgagtgataacactgcggccaacttacttctgacaacgatcggaggaccgaaggagctaaccgcttttttgcacaacatgggggatcatgtaactcgccttgatcgttgggaaccggagctgaatgaagccataccaaacgacgagcgtgacaccacgatgcctgtagcaatggcaacaacgttgcgcaaactattaactggcgaactacttactctagcttcccggcaacaattaatagactggatggaggcggataaagttgcaggaccacttctgcgctcggcccttccggctggctggtttattgctgataaatctggagccggtgagcgtgggtctcgcggtatcattgcagcactggggccagatggtaagccctcccgtatcgtagttatctacacgacggggagtcaggcaactatggatgaacgaaatagacagatcgctgagataggtgcctcactgattaagcattggtaactgtcagaccaagtttactcatatatactttagattgatttaaaacttcatttttaatttaaaaggatctaggtgaagatcctttttgataatctcatgaccaaaatcccttaacgtgagttttcgttccactgagcgtcagaccccgtagaaaagatcaaaggatcttcttgagatcctttttttctgcgcgtaatctgctgcttgcaaacaaaaaaaccaccgctaccagcggtggtttgtttgccggatcaagagctaccaactctttttccgaaggtaactggcttcagcagagcgcagataccaaatactgtccttctagtgtagccgtagttaggccaccacttcaagaactctgtagcaccgcgtacatacctcgctctgctaatcctgttaccagtggctgctgccagtggcgataagtcgtgtcttaccgggttggactcaagacgatagttaccggataaggcgcagcggtcgggctgaacggggggttcgtgcacacagcccagcttggagcgaacgacctacaccgaactgagatacctacagcgtgagctatgagaaagcgccacgcttcccgaagggagaaaggcggacaggtatccggtaagcggcagggtcggaacaggagagcgcacgagggagcttccagggggaaacgcctggtatctttatagtcctgtcgggtttcgccacctctgacttgagcgtcgatttttgtgatgctcgtcaggggggcggagcctatggaaaaacgccagcaacgcggcctttttacggttcctggccttttgctggccttttgctcacatgttctttcctgcgttatcccctgattctgtggataaccgtattaccgggtttgagtgagctgataccgctcgccgcagccgaacgaccgagcgcagcgagtcagtgagcgaccaagcggaagagc

SEQ ID NO: 13 - DNA, 810 bp, Artificial Sequence
  Synthetic oligonucleotide
  misc_feature: MHCK7 sequence
gtttaaacaagcttgcatgtctaagctagacccttcagattaaaaataactgaggtaagggcctgggtaggggaggtggtgtgagacgctcctgtctctcctctatctgcccatcggccctttggggaggaggaatgtgcccaaggactaaaaaaaggccatggagccagaggggcgagggcaacagacctttcatgggcaaaccttggggccctgctgtctagcatgccccactacgggtctaggctgcccatgtaaggaggcaaggcctggggacacccgagatgcctggttataattaacccagacatgtggctgcccccccccccccaacacctgctgcctctaaaaataaccctgtccctggtggatcccctgcatgcgaagatcttcgaacaaggctgtgggggactgagggcaggctgtaacaggcttgggggccagggcttatacgtgcctgggactcccaaagtattactgttccatgttcccggcgaagggccagctgtcccccgccagctagactcagcacttagtttaggaaccagtgagcaagtcagcccttggggcagcccatacaaggccatggggctgggcaagctgcacgcctgggtccggggtgggcacggtgcccgggcaacgagctgaaagctcatctgctctcaggggcccctccctggggacagcccctcctggctagtcacaccctgtaggctcctctatataacccaggggcacaggggctgccctcattctaccaccacctccacagcacagacagacactcaggagccagccagcggcgcgccc